European Patent Specification EP 3 630 807 B1, published August 13, 2025. Title: PD-1 and CTLA-4 Dual Inhibitor Peptides. Applicant: Leidos, Inc. The sequence listing filed with the application follows.

SEQUENCE LISTING (38 sequences)

SEQ ID NO: 1 - protein, 22 aa, Artificial Sequence
  LD01 peptide
  AMIDATION (22)...(22)
CRRTSTGQISTLRVNITAPLSQ

SEQ ID NO: 2 - protein, 21 aa, Bacillus thuringiensis
  LD02 peptide
RRTSPGQISTLRVNITAPLSQ

SEQ ID NO: 3 - protein, 22 aa, Artificial Sequence
  LD12 peptide
CRRTSTGQISTARVNITAPLSQ

SEQ ID NO: 4 - protein, 22 aa, Artificial Sequence
  LD12a peptide
  AMIDATION (22)...(22)
CRRTSTGQISTARVNITAPLSQ

SEQ ID NO: 5 - protein, 22 aa, Artificial Sequence
  LD11 peptide
CHHTSTGQISTLRVNITAPLSQ

SEQ ID NO: 6 - protein, 21 aa, Artificial Sequence
  LD03 peptide
VVKGPGFTGGDILRRTSPGQI

SEQ ID NO: 7 - protein, 20 aa, Bacillus thuringiensis
  LD04 peptide
STLRVNITAPLSQRYRVRIR

SEQ ID NO: 8 - protein, 11 aa, Bacillus thuringiensis
  LD40 peptide
QISTLRVNITA

SEQ ID NO: 9 - protein, 8 aa, Artificial Sequence
  LD41 peptide
STLRINTT

SEQ ID NO: 10 - protein, 9 aa, Artificial Sequence
  LD42 peptide
STLRGSTTA

SEQ ID NO: 11 - protein, 15 aa, Oryza brachyantha
  LD01r peptide
RTSTGDITSLRVITA

SEQ ID NO: 12 - protein, 18 aa, Artificial Sequence
  LD10 peptide
STGQISTLRVNITAPLSQ

SEQ ID NO: 13 - protein, 18 aa, Artificial Sequence
  LD10 Q4A peptide
STGAISTLRVNITAPLSQ

SEQ ID NO: 14 - protein, 18 aa, Artificial Sequence
  LD10 T7A peptide
STGQISALRVNITAPLSQ

SEQ ID NO: 15 - protein, 18 aa, Artificial Sequence
  LD10 R9A peptide
STGQISTLAVNITAPLSQ

SEQ ID NO: 16 - protein, 18 aa, Artificial Sequence
  LD10 N11A peptide
STGQISTLRVAITAPLSQ

SEQ ID NO: 17 - protein, 18 aa, Artificial Sequence
  LD10 P15A peptide
STGQISTLRVNITAALSQ

SEQ ID NO: 18 - protein, 18 aa, Artificial Sequence
  LD10 L8A peptide
STGQISTARVNITAPLSQ

SEQ ID NO: 19 - protein, 18 aa, Artificial Sequence
  LD10 L16A peptide
STGQISTLRVNITAPASQ

SEQ ID NO: 20 - protein, 18 aa, Artificial Sequence
  LD10 T13A peptide
STGQISTLRVNIAAPLSQ

SEQ ID NO: 21 - protein, 18 aa, Artificial Sequence
  LD17 peptide
  AMIDATION (18)...(18)
STGQISTLRVNITAPLSQ

SEQ ID NO: 22 - protein, 18 aa, Artificial Sequence
  LD17m peptide
  AMIDATION (18)...(18)
STGQISTARVNITAPLSQ

SEQ ID NO: 23 - protein, 18 aa, Artificial Sequence
  LD10aa peptide
  ACETYLATION (1)...(1)
  AMIDATION (18)...(18)
STGQISTLRVNITAPLSQ

SEQ ID NO: 24 - protein, 18 aa, Artificial Sequence
  LD10da peptide
  AMIDATION (18)...(18)
  UNSURE (1)...(1): D-amino acid
STGQISTLRVNITAPLSQ

SEQ ID NO: 25 - protein, 18 aa, Artificial Sequence
  LD10 da m peptide
  AMIDATION (18)...(18)
  UNSURE (1)...(1): D-amino acid
STGQISTARVNITAPLSQ

SEQ ID NO: 26 - protein, 19 aa, Artificial Sequence
  LD16 peptide
TSTGQISTLRVNITAPLSQ

SEQ ID NO: 27 - protein, 19 aa, Artificial Sequence
  LD01 TQ19 peptide
  AMIDATION (19)...(19)
TSTGQISTLRVNITAPLSQ

SEQ ID NO: 28 - protein, 19 aa, Artificial Sequence
  LD16m peptide
  AMIDATION (19)...(19)
TSTGQISTARVNITAPLSQ

SEQ ID NO: 29 - protein, 19 aa, Artificial Sequence
  LD01 TQ19 aa peptide
  ACETYLATION (1)...(1)
  AMIDATION (19)...(19)
TSTGQISTLRVNITAPLSQ

SEQ ID NO: 30 - protein, 19 aa, Artificial Sequence
  LD01 TQ19 da peptide
  UNSURE (1)...(1): D-amino acid
  AMIDATION (19)...(19)
TSTGQISTLRVNITAPLSQ

SEQ ID NO: 31 - protein, 19 aa, Artificial Sequence
  LD01 TQ19 da m peptide
  UNSURE (1)...(1): D-amino acid
  AMIDATION (19)...(19)
TSTGQISTARVNITAPLSQ

SEQ ID NO: 32 - protein, 21 aa, Bacillus thuringiensis
  LD05 peptide
MFRSGFSNSSVSIIRAPMFSW

SEQ ID NO: 33 - protein, 21 aa, Mus musculus
  myelin oligodendrocyte glycoprotein (MOG) peptide
MEVGWYRSPFSRVVHLYRNGK

SEQ ID NO: 34 - protein, 8 aa, Mus musculus
  ovalbumin (OVA) peptide
SIINFEKL

SEQ ID NO: 35 - protein, 9 aa, Plasmodium yoelii
  H-2Kd-restricted CD8+ T cell epitope
SYVPSAEQI

SEQ ID NO: 36 - protein, 22 aa, Artificial Sequence
  peptide LD01(u)
CRRTSTGQISTLRVNITAPLSQ

SEQ ID NO: 37 - protein, 18 aa, Artificial Sequence
  peptide LD17m(u)
STGQISTARVNITAPLSQ

SEQ ID NO: 38 - protein, 19 aa, Artificial Sequence
  peptide LD01 TQ19(u)
TSTGQISTLRVNITAPLSQ